European Patent Specification EP 3 848 057 B1, published December 10, 2025. Title: PLASMA KALLIKREIN BINDING PROTEINS AND USES THEREOF IN TREATING HEREDITARY ANGIOEDEMA. Applicant: Dyax Corp. Application Not Yet Assigned. The sequence listing filed with the application follows.

SEQUENCE LISTING (10 sequences)

SEQ ID NO: 1 - protein, 469 aa, Artificial Sequence
  Synthetic Polypeptide
MGWSCILFLVATATGAHSEVQLLESGGGLVQPGGSLRLSCAASGFTFSHYIMMWVRQAPGKGLEWVSGIYSSGGITVYADSVKGRFTISRDNSKNTLYLQMNSLRAEDTAVYYCAYRRIGVPRRDEFDIWGQGTMVTVSSASTKGPSVFPLAPSSKSTSGGTAALGCLVKDYFPEPVTVSWNSGALTSGVHTFPAVLQSSGLYSLSSVVTVPSSSLGTQTYICNVNHKPSNTKVDKRVEPKSCDKTHTCPPCPAPELLGGPSVFLFPPKPKDTLMISRTPEVTCVVVDVSHEDPEVKFNWYVDGVEVHNAKTKPREEQYNSTYRVVSVLTVLHQDWLNGKEYKCKVSNKALPAPIEKTISKAKGQPREPQVYTLPPSREEMTKNQVSLTCLVKGFYPSDIAVEWESNGQPENNYKTTPPVLDSDGSFFLYSKLTVDKSRWQQGNVFSCSVMHEALHNHYTQKSLSLSPG

SEQ ID NO: 2 - protein, 231 aa, Artificial Sequence
  Synthetic Polypeptide
MGWSCILFLVATATGAHSDIQMTQSPSTLSASVGDRVTITCRASQSISSWLAWYQQKPGKAPKLLIYKASTLESGVPSRFSGSGSGTEFTLTISSLQPDDFATYYCQQYNTYWTFGQGTKVEIKRTVAAPSVFIFPPSDEQLKSGTASVVCLLNNFYPREAKVQWKVDNALQSGNSQESVTEQDSKDSTYSLSSTLTLSKADYEKHKVYACEVTHQGLSSPVTKSFNRGEC

SEQ ID NO: 3 - protein, 122 aa, Artificial Sequence
  Synthetic Polypeptide
EVQLLESGGGLVQPGGSLRLSCAASGFTFSHYIMMWVRQAPGKGLEWVSGIYSSGGITVYADSVKGRFTISRDNSKNTLYLQMNSLRAEDTAVYYCAYRRIGVPRRDEFDIWGQGTMVTVSS

SEQ ID NO: 4 - protein, 106 aa, Artificial Sequence
  Synthetic Polypeptide
DIQMTQSPSTLSASVGDRVTITCRASQSISSWLAWYQQKPGKAPKLLIYKASTLESGVPSRFSGSGSGTEFTLTISSLQPDDFATYYCQQYNTYWTFGQGTKVEIK

SEQ ID NO: 5 - protein, 5 aa, Artificial Sequence
  Synthetic Polypeptide
HYIMM

SEQ ID NO: 6 - protein, 17 aa, Artificial Sequence
  Synthetic Polypeptide
GIYSSGGITVYADSVKG

SEQ ID NO: 7 - protein, 13 aa, Artificial Sequence
  Synthetic Polypeptide
RRIGVPRRDEFDI

SEQ ID NO: 8 - protein, 11 aa, Artificial Sequence
  Synthetic Polypeptide
RASQSISSWLA

SEQ ID NO: 9 - protein, 7 aa, Artificial Sequence
  Synthetic Polypeptide
KASTLES

SEQ ID NO: 10 - protein, 8 aa, Artificial Sequence
  Synthetic Polypeptide
QQYNTYWT